European Patent Application EP 4 265 264 A1, published October 25, 2023. Title: BACTERIOPHAGES SUITABLE FOR TREATING A BACTERIAL INFECTION CAUSED BY KLEBSIELLA PNEUMONIAE. Applicant: Fundación Instituto De Investigación Sanitaria Fundación Jiménez Díaz Universidad Complutense de Madrid. The sequence listing filed with the application follows.

SEQUENCE LISTING (1 sequence)

SEQ ID NO: 1 - DNA, 48812 bp, Artificial sequence
  Artificial sequence
gcgtatgaagcctacaccgtagcatctgatggcgctgaactcgttgcagttcgtcgtgctggcaatgctgcaatgcctgcggcgtaaggagccgaacaatggaaaagattatctttacgaaaggcctgatcaccaactcgcaggtggttagagagcagtggcgccaccttaccgctgaccgcaaggttttcatcaatggtgaaaacgctctggcgaaagaatacggcgtgaacgccaccgcactggtaacgaaagactactggcgcgaagtggacgacgtgaccacccgtgtattccgcaacgagtccggcatggacatgatggccgacctgatgacgctggcgaccaacatcaacatcggtaagaccgtggcaattagccgcatggcctccgatgctggcaaggttgtgcgcaccatctccggtcaggagcctgaagacctggataaaacccgctattcctacagcggcgatgtaatcccgattttcaaaaccggttatggccgcgagtggcgtgagctgcttggtatgcagtctgaaggtttcgacccgctgattgatgaccaggaaagcaccaccttcaacctgcgcgcagacatggcggattatctgctggtcggcgatgcaagcctgaatgtgaacggcgtttatactgcttacggcatcaccaaccacccgaacaccgcgcagctcaacctgagcacctctggtactggcgcgctgaacatagacctgcaaacggcaactcctgatgaaatcgttgagttcttcaaccaggatttccaggcggttctggatgcacagaacgtgttcgagccggttactctgtgggtttctccgtctgtgcgccgttccttcagccgcccgtactccaacgcggcaggcttcaaaggcggcaccattgaggattatatcctcgcattcggcaaaaccggcaatgttggccgcatcgcgtctatcggcaccaacttcaagctgaccggaaaccatttcgtcggctatgtgaagaatgcgctgtatatccgccctcgcgtcgctcagccggtatctacctatgcagagccgcgtaccacgccgcacgctaactttaacttcctgacctgggctgctatgggcctgcaaatccgtaaggatttcaatggtcgaagcaaagttttcaacggctacggcacgcaaaccgcgctgtaaaaataaaggggcgaaagccccttttaactatcagaggttatcatggctaaatacgaagttatcgccagcggaatcttcgtcaaggataaagatggtcgtctgcgggagcttgccattggcgatatcattgacgaatcaagcccacacattgagtcaaaacttcgcccggttagtgagaaaattctggaagttgcaactccgcaagaatcgcagccaaagacaaagaaaaccaagtaaaataaacccgcaaacaagcgggttttttattggggtttatcatggctgtcaggtacgaaataaacacaactccggctgacggagaggttttgcttagcgaaaccatgtcagctgactggactgcattgcaggtacagattgttccattaaactcttccggcggctatgagccattaacaagcggctctgtttccgtaatggtatcgccgtttgcatctggtgacttctggattgacgtaaacaataataattattatggcgtggcgctgcgactgaaggcgatcaagtcacaactccctgctggcgttgcatctctgaaagtcctggtatggcgatctgacacctcagtaccatcaagtcaggttgtcgcgcagtcatatgcggagcttgccaataagcaaggaaagctattcaccgcatcgcgtcgcgtgactgatgtcgctggcggggctaaccttgacagcatttttattaccggctcaaaacaggttgtgtttaatcagcgcatcattggccacaccgggaaaggtgttgtggcgtcaatctaccgtgaagccgtagccactggcggcaccgctgcggagattaataacccaaatgacatcgcgccgcatactgcaacagcgcagcttctgactggctctacgattacaagtattgggcagctgacggtggcggctacgtatagtgaagggaacgcatccaatcagggtcagggcaattcgcaggcaaaactcggtgaacaggtcatcatggcgcctaataccacctatctgttgcgcatcacgtccctggatactgcggcgcaaaatatcaatgcttacgtttagtggtttgaggatgacgcttatcttccgtgataaaagaaaagccccgataggggattttttctacttgactagtgatgcggcgtattcgataaggtagagctttggtgcaagccagatttttagccagtcgaaattattaaatatgataacgatacagatgattgaacctataccagtaaaaaccaatgccacaagaacaacttcaccatcatcacctttattccatgcaaaaatcattagataaatacatgcaataatagccattacgcaaatgatttgaatgcctgctgaagatacagcattccacatcaacagttgctgaataacatcaggaatctgtgcctgactaaatgacaccgcagaatcaatgccatcacttgccttcttcagaaggtcttccagaattttttgtgcttgttcgttcataactaaatcctcacttatggtcgcggagattgacgaggccatcaatcagccgctgaattgaggcgttgtctttaaatgtgatataaatttccgcctcatcaatatcatcaacttcatcgcccggcactccacgatttatgctattcgcaatggctattaacttttcaccatggaaagagccaaatttaatgccaacgtatccatcgccaaggcgggcaacttttgagccatcattctgagtaaaaacgccattctttttcatcactaaatcctcattggcataactgttattttttgttcttgatgtaatgctgttttgcgatatatagcatctcatcaaatgatttcccggtaacgcttcggcattgtcgatagtgttgtaacgcagcctctatggccgcgttgtcgattcctggcagtttatcgcgcaggtttttctctatgaattgttctgggttcatcctaaaatcctttttttggctatttcaaaatacacatcatctttttcaatgccgataaatcgacggccgatgttcatgcaggcaactccggttgtgccgctgcccatagtgaaatcgagaaccttttcaccttcgttggtgtacgtcttaattaggtattccatcagggcgacaggcttttgtgtcgggtgaaccgttttgttttcgctttggaaattcaattgggtatgtgggtaccctgagaactcctgtttatatattggctgatgcagcttattattaggtccgagattctcaccttgacgacccaaaaacccaacacctccacccccatttttgacaaccctatcaaccctaacaagcccttgcgggttgtagcgcattaatctctttgagccgttggccaccgccccattcgagaacaccaaaacagactcatgcgctcccattggctttagttttgccctaatgaagtctgtccgccttgtcttattccacacccagtcatatttaaacattgccagattgctgcaaactaaaatgctagtgaatggttgagtggcagtcatcacaatagcgccgtttggcttaatgatgcgcttcaattgttcacacattggctcaagagggatgatggagtcccatttgcaggcggttgtcccatatggcggatcgcacagtaccaaatcaacgctaccgtctggaatagacttcataacttccaggcaatcaccatgaattaactgaacatcttcatttataatcattacaacttctccagaatagccagcacttcattcaactccgcagatggaaggcgcaaaaattcttctgtctcctgtgctacatgaccctcagcaactaccatatgatctgcttctttcagcaactgaatcaggcggtcaatcggcttaacttttttggccttgagtgttttcgccgtcaccttatctttgccctgcgctttcgcttcctcaacggcagcatcaataacattaacggcatcatcgccatgctcacgtgcgaccgcaacggcgttggcatagctgatttgccctgcattgatgcgctgcttgatggcatcaggcacatcgccaagcgacaggtgcatctgcacatcagaaactgagcgaccgaccttcttggcgatttcttcattcgtccatccgaaccctttcaggcgcacataagcctttgcacgctcaagcgggtcaagctgcttaccctgactggatgacaccatgaaggcgattttatccgcttcatcgccggcgaagtctttgcactcaatgcgcgcaattggtacatcgcgctcaatggcacgcaatgcgccaaggtaacgatgctggccgtcaagaatcttaatgcgctttccgtcagcatcaggaataacagttaacgccgggattggctggcctgattcccagcactgcgcgaagtattcaacgtgctgctcatcggcttcgcggatgttgtaccccggctcaaggtaaagctgatcgacaggaacctgataacctttgttgaccacgattccgccgcgagtttctttgtctgagtaaatttttccgagagatgtcatcttttcctcactttgataaacagattgcgctggcaatggcgaatccgataacgattaacgccagcttgattttgaacttatcccacgccttcaggtcttctttgcggatttcgtggcggatcattgggattctccgagtgcttttgcaatggccgctttagctttcgaggtgttgacgtagatgcatgcgcgagcttctaaatccagcagtgcttccagcaattcaggcgcggcggcgatgagacgtgcatttgcgcgagtttcgtcggcttcacgatgattaacaccgtcataatccggggacaaaacgtttgcaactttgaatcgtccgcccaatcgtgttccgcgaattcgaatatatggtctgtcaacttcttccggtttaatttcccacggccccggcgtacctttgaactcattcatctccatcacctctaacatttattgttgtttctacgtcatcactatagcgacaccctcaatctacgtcaacactttatgataaaattaaaccaacaatactcaccccgcgctgttccgtcctgaaaaacgtaaggcggcgaaattggatatagcaatcggcgttatcgtcatagcgttttcgctggttcaggtgtacagatgctggaagttcatcattcggagaataattaatgagagacgcgcttcagcacgccgcaaaccagataattagtggcactgtcggccaggtaatcgacaaagccggttatacatcaatcggcactggtcttggcctgaaggtggcagagcagacgccggtcgcacaatcatacattgcctcaatgatcccccattcgattaccgagtgggcagcggtagcctctatacttggcgcgttgtcactggtggcaaaaaacctttttgagatgtggtggaagattcgggagagcaaaaagaatggcagcaccgacagcaagtgaacttgtcgccgctatggcgtcaagaggcgtaactatcaccacggcggacgcgacgggcatcctgtgtctggtggcgagcatcacagagtgccttgagcttaattaccctgaagacacatgcaggcaggatgcgattctgctatgggcatctatcctgatcgcctcaaatacagccggaagatacatcaccagccatcgggcgccatctggtgcgtcgcaatcatttggctatggcagcaagccgtggatggctctttacaatcagatgaagctactcgatacagcaggctgtacaggcgaccttgtggaagagcctgacggaagtgcaaagccgtggtttcgagttgttaccgggagtaagtgcaaatgaaaacgtcaacattaactctaaatatcgcaatccgtaaatggtgcatgccgctgctggttattctggtattgctgcgccttcctgttccgcgctgggtttatactcttgaggtcacaccatgtcagcaatagcgagatggagctatacgcagccatgcacaatctggcggcttactggcaaggataagtatggcaagccaacattcgccgcgccagaatccatcatgtgtgattatggcttcgataagaatctgaccaccggcacagctggcaatgagattgcgcagaaaaacacattctggacggaatatcagaatgcgtctgttggcgacttcatcatgcttggcaccgtcacaagtgctgacccgctggccgccggagctgaccagattagaaacgttgtgaattacggtaatacgttggaccgcaatgacctgcctgattttgcactggtaacggggtaacgtatggccgccaaaatgcgaggtatccagcaggcgattaagcgaacccaacagatagtcggagagattactggtgaaaaggctatgcgggccataaagagtgccaactttattatccgcactgaatcagccagcatgacgccgattgccacgtcaacgctgataaacagccagtatgataccgttgaggttaatggcactcgtataactggcaagattggctattccgccaattacgccctgtatgtccataatgcacctggtacactgcttggcacgaacacgccgcgcacagggagacttaaaggaaagggaaatgtatgggataagagcggcgagcctaaattccttctcaaggctggcgaaaacacacgcgagcttgtcgataaggtaatcaaaaaagagatgacgctaaaatgagagatatgcttgagcttgttgaccagtaccttagcgacgccggtctttatgacgggtggactaatcagcttgagttctggaatgataccgaagttggcaccgaccggtttatggtgctgcaatccaatggcggcacgaacgtaagcaaaggactcggcggcgattactatttttcgctctatgttgtcggccagcagggtcagtacaatatcgaggaaacaaaagcaaaagcacttgatgtcatcgcatacatcaaggaacatccagttgatagttgcattggcatgattcagttgcaggcgccgcttggccgccctacgcttacgacagagcaaaggtcggtttatgagttgttgctgagggttgtttttggtgagtaggctcgcacttaccaataagtgcatgtcaacatgatataatgcgattgtttagctaaacacagaggattctaaacatggctatttgtgcaaatgataacggcatcatcacaggtcgccagtcgctcattgagctggctgatggctgccgggatgctgtgccagcagaggaagactggaagttttttgctcccatgacctcaaaaggcgtcgacttcagcccaagcaccactacctcagaggctgatgatggcgatggctttgtcgcaacgctggtcactaccgcagacctcaccatttccggtgattttgaagttcgcaaggctgacaaggctgatgagtatggcgtgcataacctcatcaaatactttttcaccgaagtaaaagatcgtcgccagccgtcgctgtgggtacgccagaccaccggtaataccgctgtcgttgcttactgcaacattaccgccctgagctacgatggcggcaccaacgatatcatcaccggctcggttgaatttaagccttatgatggctctaccgttgacgtttccagcatcgaagatttgacgctgactactgatatcagcgcaaccaaaagcgttgccactggcgccactctgacgctcggtccggtggttgcggctggcggtgtagagccttatacctatcagtggtacaaaggcacgtctccgattagtggcgcaaccactggaactttcaccaaagcaactgctgccgctggtgatgccggtacgtatttctgccgcgtgatggattcggcgagcagcccggattacgttgactcgactaagtgcgtagtcaccgttaccgcataaaacaaaacccccgaaagggggtttatttttcctcatgctttcctcgtcttgttcttgatgccccacaaaatcagattagccataaactcctagcgctttaagtaaatggcaatcgcgtagttgatgtcaacgcgctggcctgcgtagacggatatgacatcggcatcggattggtcaacgttcatggttagcctcatataccgctctggcaaatccgcgcggtgttagtgaacgaagttgcttggttctatgggatttgccacccagccacctccagccccagaacattccaatatttaccgggcctggatttttctctggcattacaaacccgccaccagcccaaatgcaggtctttttcgtgtacccgtcataagctggcatcttcgggtgaaaactttcctcgctgccgtccatgtaaccgccatactcatacgggtcgaagtagtaatccggcttgcgccagagcgttgacatcttgcccaccgggttttccaccacccaggggattccgtagcgcccggcgattcgctcgacaagacgagcgctatgcagggaagctagtccttcatgtccatgctttgcgccggatgaggcgaactcagtgcagtcagggaaggcaaagataatccctggggctggaattcccatagtccgcactactccattaaacaggtcatcaatccagatatttacatagtgaatgttgctatgcttaacacgaattgactcataatcgccatgattcgcgccatcataattaaagcagtagcattcatgccctgcctcggcccacggtttaaccataatccctgagccatcaaacatcgaccagaccaccatcatgcgcactcatccagttgacggcgcaacatacacagcgcaccatgcggcataaactgcgaaaccattccgtcgaatatctgccggtttaatttattatcaattcgcggcctaattgcagaccagcacgaccgtatagcgcgattaacctggcggcggtcgagcattgcgagtcgcgcagctaactcaatggtaacgagcgcgtcaagatactgctcgcatgcgtagcggctttcattattcattcttagagccttatcatctggtgtaacgcgtagcgtaatggtaagaatccatgcaccatttagctgcctcctgcctaccagttgttgtacctatcaggataatgcttacagtgccatctcttgagttgcgctttgacttaacctcttgcatatcaaggatgtcgccttttttgagttcgctggcagcaatgtacatctctcttcttgccatcactcaccctcctgcatcatgaggaagacaatcatggcggcgcggagtgggtttttatggttcacgcgatgtttaacatatgcaggcttgaattgcgctcgccacgttttttcgtgcctgttcaccacaatacattccagagaaatgccattattaacaataatcggccatgcatctgctgggttgttgcagtagtcaaaaaattcattagtgccattcaaatggaacacctgaacatcggggcgatgattgtacggagttgttgtttgtgacctgctgtaaatcaaagaggcaacagccttattaatctcaaaatcactcatcttgctgtaatcagtgctcatctcttatcctccaccactacgccgaccttcgccagcaacaatatcgcctttacccgagcctcttcatatgtataaccctggtcgatgtacaggtcgatgtaaaatctcaaatcagcatctgtttcgctcatcttatgcgctccttatggcttacagaatcaatctacgtcagttttgcaccccctgtcaatggtataattacgtcattgtgaaaacaggatttagacatgagacaacgcacacccctaacagaaatcggagagatgcgcatctccctggctgacaagtcttttttcttcaaaccatcatttgcggcgatgaatgagcttggctcaccgaaagagattgtcgagctgtacgctacgcttaatggctatgaatacgcagccatactcggtgccattcagtcaatgccatatggcgcgcagattcaggtggcaaaaatcctgtcacgtcctgcctatggcaagaaagtgctcagcgccgcatgcctcatcatgcagtcctgttgtgatgatgatatctcggtgctcattgggtcatggaagccgactccgcgcggtgtgaagtatattcctggattgataccaataggaggaaccgggcatctccctaatggaaatgctggaatcattgatattgctcgcgcattaatagagcatggcatcatcggcaagtctccgctcaaggttcctcagcgctcggaaaaccaaaagcgcacaaccagtgaactgagaatgtcggattacatcatctcagctcgcactcatttcggaatcacccgcgaggaagcggaatacctgaccatgaccgagtatcagcaaatgataaaatcaaaatacccggaaccggaaggcatgacacgcgagcagtatgatgcgtcttatgaacgggccaagctgaataaacagaaactgaaagagaaagccgccagaaaggccgctaaagcaaaggagcgaaataatggctgaagaagttggcggcattgtctatgaagtcggcatggaagtgtccggccttactgctggcgcaaaacaggctgaggacgcattaaataatatcgacaaatcagcgcagacgtcatccaaaagcatggataagcttgatggtgctgcatcatcttctggcaaagagctttcagcgctggcaaaggtggtcagctcaattgatgccaccctgaaagacatggcgtcagcatcaaaaaccgcagctacatcggtggaggaaacaacctcaagcgctgtaggtgcagagcaggttattggtgcgttaaatcagcaactggcgcagatgcagcaggcgcaggtttccgcaaacgctactggccttgcgctccagaactcagttaatcaggtcactcaggctattcgtgctcttggcgctcagtccactgaaaccggcggatcgatatctggtatcgacaggatgattgagtctcttgggaatcagatcgccattcttgatgagcaggcagaaaaaggcgcacgtagcgctgccattcttgccgctcagttgcgagctggagacagtgccacggatgcgcaaaaggcaaagatagccgagctaaccggtcgactctatgacatgaaaaatggcactgaggctgccgggaagtcaacgggtaactttaagaatatcatgcaacagggcggctaccagattcaggacttcattgttcaggttcagggcggtcagtctgcgcttgtagcattcagtcagcaaggttctcagctggcatccgtatttagtcctgttgccggtgcggtgctgaccatcgcaaccgttattgctggcacgctcattgcttcccttggtgacggcaaaaacgccgttgatgcgctgaaagaagctattaccacaatggatagcgtagtgtcggtgtcgtcttctggtgtcgcagtatacaccgacaaattcgctcagcttgccaaggtcaatgccagcgtagcaacacttatgcgccagcaggcgcagcttgagttgcaggcagcgctttcaaaagtatcagctgaagtcaccaaggcatccagcgattttatcggatttggtgattcgctcgtatcttctcttggtggtggctatgccagtgtcaagctgttcaatgactacatgtcgcagctgaatatcaccactaacagctggacggaggctattaagcaggcatctgcggctggacaggctggacagacgtcaatgaatggcatgattgctaccgttggtgcgctggcaagcaaattccagctttcagatcagcaggctttcgagtttgcaaaacaactgtcagacattgccaaaaatccatcagatgaaaagctacgggctctggtggttacgctacaaagggtcggcgagggaacatcaagcggcgctgtaacggcgcgggaatatgccaagagattgctggaaatagcaaccagcagcgcagatgccactcagcgcttacggcttttaaagcaaatgactgatgagcttactgactctcaggataaggcgcttcagcaggctaagcagacgcttttcattgagcgacaaactggcgttgaaaaacaaaaggcgcttgcatggcgtgatgcagagaatcagggattgaaggcagggactcaggcattccgtgattattataatgttcgccttcagacgtatcagcagcaggagaaaaatgctcaaagcctcaaggatgaacgcagcgcacaaagcgcatctcaatcagcagccaaaaaggcggcgactgagcaggaaaatattgctaacaaacttgagcagttgcgccagaaatcccttctttcagccgactccaccagagagctaagccgggagcagtcaatccttgcggctcagcaatcactcggtaaaggcgcgacagaggaacaaataaatctggccgggcaatatgcagcaaaagcgtgggataatgccaatgcgctgaaggcgcaagctgaagctgagaagaagagagttgaagcggtgaagggttttgccgcccttaaatctcagacatccccaatgtttgccgttgaaacaaattaccagaaggatttggcagcgcttaatgcttacgcagtggcttacccgcaaaaagtagcagaggttgagcagaccagagcagccattgaggagcaataccgccagcagcgtcttgatgctatgtggcaggagtggagccagcagaatgccgccactcaggcagtcgcagcagcattcgaggcttttggtcagtctgccagtaacgcgctgactggtgtcatcactggctcgatgtcgctcagtgatgcactgcgttctattggctccaacatccttaacagcgtcattaactcattcgtacagatgggtgttgagtgggctaaatccgctatcatgggtcaggttggaatgactgccgcgacagcagctactgccgcacaggcagccggtatcgctgctgcaatggctcctgctgctgcaatgacatctcttgcaactggtggcgctaacgccattccagcacaggctggcatcactgcaaccgtcggtgttgctaaggccatgtcggtagctggagcgcttaaaaatggaggccctgcgcaggctggctcaatgtatcgcgtcggcgagaacaacctgccagagatattccaggcttctaatggtaatcaatacatgattcccggcgatagcgggcgagttatcagtaacaaggatattggcgggtcatcaggtggcattgtgatttataataatgtcaccaataacagcagtggcgccacagcaaccagcacggcgcgagataatggagatggcactgtgaccattgagactatcgtggcagacatcgaaaatggcggcccgatatcgcaggccattaccagcaacaccactgcaaccagaagggcaacagaataatggctatcgcttacccatcgtggctaccgctggcgcaacgcgccagcaaaaacatgacgactcaaacgccgttccgcagcgatcagcctgctgttggcgcgcctatcttccagaagctgacaactgacgttgcagtaacatggagcctgacgtggatatttacccttcggcaggagcgagcatttcttcaatggctgaggagcccaaactatctcaataagtgtaatgaatggtttacaatggatatcgaccttggcggcagcggactgcaaacgcagaccctgcactttaccgattatccagtacagaccagcattaatggcggccttgttacatggacgggcaatgtcatctgcaagactctcaataactcaatggatgagtttgatgatgttctcgttgagcttgatgagagatggtattcatggctggacgaggtcgttaaccgagacttgccggagtatccataatgccaacattacgtgaataccagtcaaagcgcccaaactggaagctgtatgatacgataactttttatcattcttcatttggatatgtccggcttgttggcaatgagtttgaggatgtcgttcttggcggccagacctatcaaccggtgaggatggatgttacccgcagccagcaatcgaacacgccggttatcaacgcaacgctgaagtttgcgcggctggcaaatgactttaagcaatatctgaagctctggactggctctggaaggattgagccaatcaccgcgctttatcagcgctttgatgaaactgacaagaacacgccgctgaagccgtacacactttacgttaacgatgtgacgcttgatcagtctgatgtgactgtctccatttccatcaaaaaccccattaacggcaacgtggcaaaactttatgacatcacagaatttcctggactgcgcacagtttgagttgcttatgcttggcaagccatatattgacaggtgttgccatgaggatgcagtggattgctggggtcttgtggttctcttttatcgcctttgtcatgggataaacgttcaccacgacgattcatattcaacgggtggtgactttgtcacctgctttgatagcgaggttgcattctggctagaaaccacgacgccgaaagtcggtgacgtagtagttgcatatcgcggaagccatccggtacatgtcgcgctgtggtggggtcgtgataaaatactgcatgcgcgagaaaagacggcggtcaaaacagatcgcctgcgaacactcgaaaaactatcaacaaaattaaggtttctagcttatgccggtgattcacattcagaaaatgccaggggtgccaaaggaaactggtaatgtggcggttggtactaacctgtggcgctggcttgaaagttctggcctgccaactgatatccgcatagcgctcaatgggcgtgtttttggccctgatgatgaattgtcgatatcgttaaagcaaaacgatattattaacatttactgccagcctcgcggcgccattggcgaccttatcagcacgatactcaagcctgtaactaaggttctttcttttctgttgccaaaagcatcaacgccatcaaccagcactggctcgacggttgaatcacccaacaacagcctgaaatcgcaaaccaatattgcgcgaaacggagaggcaagacctgacaacttcggtcagataagggcattccctgacctgattcaggaatcgctttttgaatacattgatgacctgaaatatgtcactgagttcatgaattttggcctcggtaaatacaccatctcatctgttcgttatgcggaaacaaatcttggttctctgcccggcgccactcatgtcatctacaatccaggtgatgtgatcgggcaaattattgagccttaccagttcgacgggcttgatggtcaggaggttccagggctgagcgagtcagaggacaccccgatagagacagcgaccacgacatctgttaccagtggtgattatgctggcggtcagctgttaatggtcataccaaaaaacactgatttcgattactttatggggctctctttaccacactctgtgtcattaacaataaatattacctacaactcgacatccgggccagttactgaaaatatccagcttagtggcaacatcatttcagctgaggaaactgagacaggcgtcattcctgatattcagtatttctataatttcaccttcaataacctgacaggcgcaaatcttggcaatctgactggcgcaaccatcaacaacacttatttccagattgtggatgatgaggcgctcgttgttggcccatatgttggggctgtggaatcaacgcaggtttgggttcacgttcagtctgagcttggacctaccagtggcacggcagattatctgatcaaggtatgggcggttgatgacaatggggatgctattcccggaaccgaggagcagctcgcagacagtattgacaacccatttaatcagacaacaaaaacctattatcgcacgtataagttaactcctacttatgggttggctaagtatgccatcagcattgaaaggacaaacaactcaaactctggcaaccgcgtaacgttgcaggcggcgcacgccatcaacatccgcgagaatgtagtttatcctgatgacacccttgttaaagtcacggtgaaggccacgcttcagcccacatcggttactgagcgaaaatataatgcactaatcacccgctggacgattggatataacagagcaaccggagaggtagattacacattaactccatcaagaagttttgctgatgcagtgctgcacaactggcttatcactgccggacaacctgagagcaccatagatattgcaaggctctatgagattgcagattccctgccagatgcgcgccttggatattttgactacacgttcgatgatgaagataaatcaatcggcgagcgaattcagactatctgtgacgccgctcgcgtcacagtattctgggatgatggcgtcctgtctttctcgcgtgatgagcaaaaatcaacgcctgaaacggtattcaataccaggaatacgcaggcagatggctacaagatgtcatatgatatgacccttccaggttcatatgatggcgtaagcgttcagtaccgcgacccaaacaccaacaaacaggcttacgtttattataaagttggggcatctggtatcgaaccgggagagccaactaaaccgaaaaaattcgacatgctatacattcgaaacctgtatcaggcaacagaccgggctatgcttgagtgcaaccgtctcatgtactcacgtcgcggaatggagataaaggcgcttgctgatggcgagtgggtaaacgttggcgatatgatttctgttgtcgacatttatgattctgtacagcagactggcgttatccgatcaaggtctggaaacgtatttaccaccagtgaacagctcacggcaggaagcggcctgtttgtggtcatcactggcgccaatgggaatgtgtcagaacgtctggcttgtaccgttactggattgaataaattcgagtgcgcattaccatctgacttcgagttaaatatttttgacggtgttaatgttcagtcagaatcaagatatgcaatctccacggaggttgagcttgactcaactttatggacagtcagccagaaaactccaggtacagatggcacagtgtcgctgactgtaaccgagtacaacgatgccatgtacgcctacaccaaccctgttgcgtgatacaatagggcaattaatgattacggagattgcagccgatggctactaccccaactaacaagccaatcccttctgaagacccgcgtgacctgaagtttaacgccgggaagattgatgaagaggttaacggaagttctgattactacaccgaccgattcggcgtgcagcggctgacgaataccggcaggaataaccagtttcagacagcacaaggtgagcgtgaggcagagtttgttgcgtcacaggtggataaagaagcgcgatttcaacaatttcttttaaattctggttatcagtttttgggcgattacgaaaatggtccgtatacaattgccgccagaaaccagattattcgttatcagaacgagttctggcgtttaaacgcggctaccaccccaccttatacaactacggggattaacagcacatcatggacggttgatgtcactcatttagtaagtgttggtgatgcttctttaaggcaaaatctgtctagtgataacgggttgggtttgataggtcagtgctctagcttaaacgccatgagagaaattgagttttcatctgctggtaaacaaatattcctcaaagaacatactgctgggcagaatgctggtggtggtatttggtattgtcactccctgacgtctgacagctcatacgtcgatgataatgggtgccagattatcaacgattatggacaggtcatccgccgtaaggatgttaaagaattaacttcaagtgactttggattgaaagctggtgataccatcgacactgtcctcactaacatgtacaaagcttctcgtacatttaacatttatgaagcaaaaattgaaaaccccggctttgataaagggtatgtattacaaggtggtctccggttttactgtggggataagcctttttatatccactcttattccataagtacgttacgaggaccaaacctttggcataccgggaataatgtcggagttacgttcacccgtttcaaagaagacggtacgtcacaacaagcttggtccggtggcggaatcaagggcttccgcatttggggcgctgcatcttaccttgttcaaggaaataccggtgtggatgctacaccagtacgcctgtctgatatgtggcaaggagaggcttgcgacttgtggattaccgggtatacggggaatactaatggtgcatcggtttctctatataacgaatttgcgtggacggaaggatctcttgttaaaaatgtaatggttcgccaatcactgcgtggtttaacatttcttcgcaagcatgggactacagctactgattcatttttccgaccagaagttgatttttcatttaacgctggtgttcctgggaaatcaacacaagtcatggttgttggcgatggaactgccgctggtaaatgtcttgtatacggccatgatattaagcttactcagtggatgagtgccggggcatggcacgatatcgtcaggcttgaggactacagtattatcgcggagactggagttattaaaatagttgcagatggctacggcatatccaaaactactgtaccggaaaccgaggttgttcactacattaatgtgcgcggactcaatgcccggttccggagcagagtggaaaactggtcgaatcaggctggtggttggggtctggatttcctgaacatcatcttccagtccagtatgtatactaacgccatgacgttttatgagtcggattttgacgcgctgccaaccattaaccccgtcgggatgaaggtgcggtttaatggtacgttcactgttgctgagaggcagtctggcaaggtgtacactcttaatgggttgattccggggatgacactgaaagtcaagctgacgtcccgcaacggtaacgaccttaatgatgctgttgttcaggagtggaaggtgtttgttcgcagtaccaacttcccgtgcatagtagtccctatgtctggtagtgcaaacattgctaccaccgatgggttggctgtcactaatatcagcccagtgcagactgctacgttccttaagacggttacgcctacgcaggctaggaacttcatcggtcagaactacggactcactgtgaagaacgcgaatgacgataacagcatatcctatgctgtgaactcaggtcgtaatattcgctttattcttccagctaaccctggggcgactacgacatccccgtactctgttgagatagaggtactttaaatggaaagcaatgttgaaaaaatcatacctgtatttgcgttaaaaattgcaagtgtaggcgagatcacagatggtcagtgcacgttaactttggaaagtggtcaggaagtttcagaccctgttgttgtgtcagaagagtacgtgcaaaaatacgaccccaacctggcggctactacataatgtgtgagaatggactcggattgtactctaattaaataacattaatttaattatctcaaatgaaaaataactttgacaataagcgcatcaattgcgatgcgctttttacttaaaagtcaaaaaggaatatcatcgtcaaaatccatcggaggctcgtttgccggtggttttgacgtgtttgatggttgctgaggtttaccccatcctgtttgctgattgcttcctgattgttgccgctgctgtgatttttggtttccattatcacttgatttaccaccaatcatttgcataacgccgttcataggctgcaagacgatttcagtagtgtatttttcaacaccgctttgatctgtccatttgcgagtgcgtaatttaccctctatgtatacctgagagcctttgcgcaggtattcgccagccacctctgccagctttccgaagataacaacgcgatgccattcagtttgctctttcttctcacctgtggccttgtcattccactgttctgatgttgccagagaaagattgcacacagcgccgccagaaggcatatatttaacttccgggtcttgtccgagagtgcccaaaatgattactttgttgattccgcgagatgccataatttacccttaaaagttttcgatgttctgttgagatgttgatggcttctcttcgtttgcagatgacacgggcgcatctgctttctggagttttgccgggttgaaatcgtcctgcggtgtaatagttaccgctgctggagattcatcattaatgaatgattcaatgcgctcatactcttctgctgatgccttcaatgtaggccagattgtacgaatttttgctttcactgaatcaggcaagttaactgcctcggcagttaacgcagcaacgccttttgacgccgtcatttgaagtttagagcgccagtgctcaaattcttcgtcgaccttgacacctgaatccacccatttaattaaacctcgcccatgagcatcgcctaaatatccttcgtgtacactatcacggcctgaatcaaagaaaattgggcgcaactcttctggtagcttggtaaattcctgaatttttccattatcatacatcatcatgcttactgtcatttcaaacataaaatctttttcgcatacagcatgcaatccgagggattcaggtttcttggggtttttaaagctcgttttctctctggcgcgtaaacatacaatgatatgcatattgctctgtaaaagagcgctcatgaattttttatgttcagacttggctcgcttccagtccgccattgccttaccttgcaatagtggttgctctgcaatatcattgcatcctccttcaccttcccattcgtgcgatcctgaatcaataaccaaaaccttaacgcctgcctcctgaaattcctcgatagcctggcggtaacgagctggactaaatggcgcatacaaatcagcgtgcataaatggaccgtcaagctctccagaataaagcctgccacgaccattttcagagtcaagaaatccaatttcttctggtttatcgaccatacctcgtgccatctttagtgccgtaagcgtcttaccgctaccagactgacctgaaatgccaatcactacgcgtgaaccagagcgctcggctggcttaatgtttaaaacacccatcacttcacctcatttactataaattacatgttaaattgctttttgaaccattccggcgtttccatttcgatgaccggattacccattgagtaaccgggccatgaattggcttttttgcatgccttatagatttccatcgcgctgcgcagctgaatgcgaccaatgcgtaactgctcatccgtcaggcgaatcagcgcagggatgaatggggattttttctcctgcaccagaagatttacagagcgcggcgcatgcccgtaagcctcgacaaacatatcgtgttgcatcgccatcttcataaagtacccgagccgcgcagcatggcggaaaaactcatcaggcttggcgctcaccgctgttttgtagtcaatgatgtctccgccgcgtgtaaggcagtcaaatcgcaccttggcaggctcgccattgagttctccaaggatggacacctcagtatatgcgccagccagcaagctgctgtaatagctgtttgcgtggattacggctctcatctgcatgattgcgtcataatcatctccttccagcaaaattctgcctttcgcattgagttcagcaagaaggcgctcttcatcatagattctcactggttctccagttgagcggatgattttgataacctcagcctttgtcttgccagaaagacctttgattccgcgctctttcgcccatgagttcatgtcgctcacggtaacaaggagattatctccaaaatcatctttcgtaggcatgcgagcatattctgcatcgaagcactcaggctcaagcagagctgtatggctaccagtaccgaaaacaagcgctttcgattgctcgtcttcttcatccttgtaacgccatgctgctgggcatctgtcatacagattccacaagccagagccgttgatgtgctctgtgtcagcatggtaatcctgattgcttaattcattgttaaagtaaaccttcatccatcacctcacttgttattgtcaaatgaatctacatcaaaccacgtcattcatcaagcccaaaatagaataacgtcgctttttttagctcatcaagaccataagcaatggcgccaaagtgaccctctgagatagcctcctgcagaacctcaatctgcgatggcgatacttttgattttgtcttatcacgccgcttcagctcaatcaggccgcatttatgattaatgccgtgcgtcagtatcacgttatcgcttacgccgcttcttacccccattctgcggcgtttttcgacgaattgcggtccgctccttgttcctgtctcgtttggaacatgaaaccaaagcacatccgggaaacgatgctgcatccataatccgtagctaatctggtcggtttcctctttcgggcaatctccacgatagccgctgtcaaaaacccatatcccgcttttaagctgcttcactctgctctcctgtgaaatccttcctgtggatgatatcccgccccttatcgttaaaccggtgagtgatgcgcttcggcgcgcggataagactggcataggtcatgaaggtttttgcattctggcaatccatcatctttttcatcagcgatttatcctccagatgcggcaacaaacccttcattttaaacatatcacgcaggtgtttaggcttgccgccgaaaggataaaatacctcattggcccagccggttttgccgtcagctttcacgcatcggtagcgatatagaatgccttcgccgtcttttgtcagttcaactttaaaatcctgaacgtcagtccattcattatcggtgtacgcccgctcattcagcgccgaattagggtcacgcagcacatggtcgcaacagcggcaatagcgcgctgtagggtcgtttttaactccacaaccatcatcaaaaatgcggattccgtgcttatcaaaaccgcaccggataaagctaaaaaactcctcgcaacgaccatctgctgaattgtcatctcgtccaatacaacggcgcgcataagggctgttcatcgtctggcatttagggcatggaacctgctcaccacttcgacttgatcgctgcgcttcagcctcctcaagaatagggtcttcatagaggctccccagctcaaacatggttccagtgaagtcaaggcaaagatgattttctttaatcaatcctgctgcaatctggtcaggcttaagcaggcgcatagggcgtccaagcaactgagtcagcaacgtaagtgacataatttttcgcaaaattacggacgtatcccagtatgggatgttaacgccggtggtgaggcaaccgatttgcagagtgtacttcttgcgcccggtagccgcatctttgagcgccttgcgtctggctttcatgcccatgtcttcggtgactattgaatagctaccctctggcaggtattttgctgcttctttgcagtgctttttcccggcgcaggtaatcagtacaccaagtcggttttttgtcagttccataacattcaacatgattttctgtgtcagcgtgccctgctcaaggatttccttctccatctgcttgagttgcgcatcggtaaagtcctgcacaccatccacgccactgctttcaaattcatgcaggtcatattgcagatcgtcaatgtcaggcatcccgaaaatagtaggcaccagataacctaggtcaaccagatatttggtgctgatgttgactatctcatgcttccagtacgggcctttgatggaatcagtgccacggaacgggctgccggtgtagccgatgacaattacctcatgtccatacttctctttgcagcggcggttaagctcggtcatgataacgccgtactgcgtttcaggatgatcgcttacgatgtcctgccagttaacctgatggcattcatcaaccagtatgtagcgcggggaaaagtctgatagcagtgatttcgtcacggtgccatcatcggatgtcttatcaaaaagaccatttattattgttccctccgttcccgctataagcggataggcatatgctttacgcccaagtgaagcgctaaacagagagttttttacgctcagattccagagttcctctgcatcctgctcaataatttcgccttgtcgcgcgatgacaagaccctcccatcccatatcttggaaacgacgggcaatcatggctatcatgatggtcttaccggcgccaactgaagcggtaacataacttggctttggctgcttaccaaacttgcggataacctccgctgtcttttcatataccagccactgataggggcgcggttcaattcccccggtatggatgctggcccgcagcttatccatatccagctcagcaatcattgcatcaattttttgcattttgaatcacccaattatttcaatcgcccaaaatctttgtggtattttttagatgctattgcatacgccattgcggctgcttcttttgtggcatgccttccaagccatatttttttattattaacccatatccagcaagtccatctacctgtctgcttgcaaaaacctacacctttcactcctgatgtgttgtgttttggggttctcatgtttctaacattttcgttaaagtttgcctctctaaggtttcctattttgttgtttaatggattcccatcgatatggtctattattaactcaggccaataaccatgcactaacgcccatattattctatgaacctttatatcaaaacctaaaaaaccaacctgaagatatccacttacagtctttgagcctgcaatagcaccacgtttcaccctgtttgttgttgttcttttccatatgagatttattccgtcatatgaaaaatactcccgcagcgtggatactggaattgacctctcttttgacttcatcaattcgaaatcattcactttacgttaccctcattcagtgttacgcttaaagcatacaaacagtaacagatggagtcaacatgttttattgggaagatatacgacaaaggatgattggcaactgggaggccgcgctgctatcaatagtgaatattgacaggaaggtttttaatggaaagcatcagccttgccctcattgcatgggtaaggataggttcaggtgggacaacaacttcgaaacaaaaggcgacggtggcgccatctgcaaccagtgcggaaacggcagcggaatcacctggctaatgaagctgtcaggaatgacgtttccagagtcaatggaggcactggccggatttcttaacatgcacccacgcgaaaaacttgaggcgattagaaagcaacttccgaaggtcaaccatgcttatgactacctgacagaggcagaagtggcggccatcatggaaaaagccgggggcgacacaataaccggcaaaactggtgaactggtggcgataccgctctatatggctggaaccatgtcgccgtgcaacgtggcttttctggcagacgatgaaagcgtatcatttcgcgcaggtttcagccaggagtacactcgcggaagacttacgcgaggtgcagtgacacccatcggcgataagactgaatggacatacctggttgcggattacttcgatgcctggcgagcgcatcggcttaccggcgctcatgtctggtgctgctggtcgccggaaaatatgtgggaggttgtgcgcaatgtgagcgatgagcagcgggctaaactacgctgtatcattaataataatttcgatgaggtatgcgccgccgagaatacaggccttccaatactgattactgatgacgggcaggatattcgttacagtggcgcaatcagaaaaaggctgtataaaccagaagaactatttgaagcactaaaaaacaaaccctcctgatggagggtttttgttcaatacaaatcttcgctaaaaagttcatcactaggccatgtttttattcttactacatttaactgacctgcatcccttgcaacctgcaatgcctctttcctgtccataaacacaccgaattggtcaacaaacccctgcacttcagattcacgctttatgaaatccttatgtggctccatattctgacgcattaccgggcagaaatgtctaacacctataaaaaccatatcaatcccaccgtatccgcaatcatatttatttgctgcgcatacaactcttctttgtaatctattcatcatttaagcctcggattcaggtaaacagtattattgaggaatacgcaatatccatcctcttcaagagatggcaaaacgtttgacttgagtctgtcataaatatgcggtatacctttgaatggtctaacgttttttagtgaatcatacagccatttcactgtgacatttgtctttcctttttgcgcagctgtgcgcaatttctcagcaacaacgtcaatttctgatttctcgccagcgtatccatttgactcaactgcatcggtgaatgtttttgtcaatgcatcataaacgcttatggcgcggcttatatgctcctcaccaataatttttgagcgacgaccgccatcgcaccagttttcagcggcatggaatattgccgaaagtctgattatctgtttgtcagccttacccatggcgccacgaagcaaaacgtgatcccattttccacctggcaggaaattcttttcccactggtttcgtaaaagtccaatcatacgctgcgattctttagcgagggagaaaacaaccttctcagaagccacaaggttatgcacaaatctggcatattcagcttttaattcttgtggcattggtttgcttaccggacaatcattttcaacatcccaatgctcacgataacccaacattgactgctcgcgaagcatcaggaatcgctctgacaacccgttacccctgtcaccagccgacagaatggcatcaatactttcatcctgtgcaatgacgctgatgttaccaagaacatagccagatgaaacaccacgaccaacgcgagctgaaccaacaaacccaccgtcccagcctttcaggatgacctctgcgttagactttccaccatctttgccatatgaaaggccaaggcaggtatttaaaacgcttgcttcatcacttatcaggttgaaaaatccaccttcatgaattgcctggtgctgcaccgcttcaggcgttgcatcggttaacggatatgtgatggtataaagactttccagcttttccttttctttcgcgatatcatctccaatgatggctttcgcgttctgattcgtcgcctccttgtaagccttcatcaggtcttcaatgcgaatgtttatttttacaatttccttctccatcttttttgacaggttgtcatactcaatttttatcgggttcatgtgcattgagtttatggctgtctttcccgctgatggaggctgtgacgtcaccacatacaaggaaactggtaactcagagccatagtattcaacgctaaagtttctggtcatggcacttgctacgcagccaagcagatgcatgaatgacgtgctaacggggaattgcacagccctcgctgccgcaactgagtagcgcgttatcaggtctttcctgttgtcactggtaagctctatctctgagtatgttacatccttctcctgaccctccttgatttccggccacatgttatggcttggcgtcatgccatggtgaatggctacgcgcgccgcagaggtgtgcgcttctcttgcctgattgaatatttcctggactgcaatcatttaaacctcgaattcagtcgcaaataattcgtgagggttttctgacagccatttctttgccttcagaacagctaggttcgcttcttctgcggtgtcgaacatgccaatgtcatatctctttttgagcaccataacgcgcgctcgaaatttcttcgacgccttgtgatagtcaacgccgtagtaaccagttgtagaccttggcgatgcgacccatctggcaccgatgcgattatcatttcttttccgtttcaataaaacgccgtgattgctcatccaacttccctccactttatttccctaaaagataccagaagattccccagcacgcaatgatgctttcatttaggcggatagggttaactggggcaggcgtggggcatgccaccttccccacgcgctatctatctaagtgtatgtaatataataataatagtagtagttgggttaatgggtattattattactcatattatagagtataatttaacatttaattaacatatgtattattggatgtatttatagggggatacgggtcaaagttaaccaagttaacccaaaaaaaataaatcaaataaaaacatgcaattaatacaaaaaatttggggcaactgacttgccccacgacctgccccaggggcaaaaaactaccccacgtagacattttttcatcaccttattgacgtagattgccatgcattgtatagttacctcaccaacaataacgaggtgatgaagatggaacaaaaaccagcaggccgtgtggtatacaagcgcactcatctggagcctgaatttggcacggtgaaggcgcaaaactttatgatggcacaggcaatgcatgcatacagcaacggcaagcgcgtctgtcgcgtttttagtggcgaaggcaagcagagagtgcttgagcaggttatcgtgtcatctggtggaaactaaaccggtttagcaacgatgaataaattactggcagtggttctactggttatcgctaactcagcaagcgcggaaacgatatgggtaacgaagtacgcgctgacccgtggcattcagaagtacgaaagcgcacagctgtttgccgatggtcaggtggctgtggttggcgatgtttactttaaacgtggtgaatactggcttgatgagcaacaggcaaaagagcatgcagagactttgcggcagcgccgtgtatctgcattgatgcgtgagcttgagcgcttacaggcggttaagtgaggatttatggatatcgaaattaacgaagttcaggaaattattaaaagccttgagagtggtggtgaactctcaatcaaagaggaaaaatacctcaatgttgcaaagatgtgcgtgcagcttgctgcggagaatgtggctatgcgcaaaacacttggtgaggtggtctattcatccgaagaggtagagcatgacggatgccttacattcgtagttaatcctgactgcgtgcatgatgcggctgatttactggatggagaaacccccaccaccgatcgcatcgtagccgggattaaggctgatggtcgcgcagagggtatcaactttgcagcaagccgccttgctgctgctttcaatcacggattcgttgataagccaatggcagaggttggtgacgtggtacgcatgatactcaccgcaaaagaggatttggcgaaagacccggtcttagccgccgatggactgtcaggagagtacgcagaaaaatccctggctgaatgggaagctgcgctgagcgatggggccagctatgactgatatcaccgaactggcgcagagcctgaaagcggcagccaatacaacctccgatgctatcgaccgcctaaaagcattcccaggcgacgaactaattgacctttcacagcatgagggtgaacaggtagacattgatatcacaatgatcaatgagtggtacgagctatcaagcccggcaaacatcctcgcgctgctagaggcgctggagaaggcgcagtccaaaatcatcgaattgcaacagggctacgaaatcgatccgcgcaatcacgaaattatcgacctgcatgagcgcatcgccgagctggagtcccgcaccgtgaagttgccagagctatgcgtgggggttgttcaaggtggacatgcggtaatggtgccatatccagcaggacactggtttaacaagacagcgattttggagatgttggccgccgctggcatcaaggtggagattgagtgatgtgggtgctcattatctggatgttcggcggttacgaaaacccgaccattaccactcaagagtttcaaacagaatccgcctgtcgagctgcatttgccgaagtgaaaaaggtaaacaatgccgacgtttctctacgtggcgtatgcacgcctaagggtgaccaatgaccaaatcaaccataaccagagagcgcgcacagcaaattttcctgggcaacggaccagagccgagcgcatcagaagaacgagagctggcccgcatggcgctggccgcaatggacagtgagccggtgtcacaaaatgagcccattagttttgacgagtggtcacgaaaatgcgctttgcaaatcacgctttgcgaccctgattttcgtgaaaaggctaagtacatctgggattcagcgcgcgaaacaatgcatccagcgccggcatcaatgaaagaccatcagattcgtgagttggtaaacgagctgcgcgatatcgctatcgagcaccacagcacgcagcagttacgtgaacgcattgccagaactgtacgcgccgccatgctcacagccgtccagcagtcacccggcagagagcccgctaccgtgccgggtacatggattccggtaagcgagcagatgccggaaattggcgatatcgtgcttaccgcaatgggaggtgtggttaacgttggcgaaatggagtgctctgctgcaaattatcgtttcttcacgtcagttatttccggccgcgagttaccggcgactcactggatgcctctgccggccgctccgcaggaggtgaagtgatggaatggtatttctccatcggtcttgttttgtggattttggcgcaaataacaagagcagatgaaacaactggcattaagaataacattctgtgcttgctgctcttcatcgtgttgtggccaaagatcattatgaccattgcttgcaaatttatcgaggaaaatgggttgatgtctaagtcatcagcagcagtaaaatccatgaaaccctacatcatccgcaggattattgccgtagcctgcattgcattctggattgctgttgcactggccgtctactttatcttgaggtgaatcatgttgtggagcgacattcaagctgcatgcgaagaggctgattttctgtatgaggagaccggaaagcatcatgctgttattcaggtaggcagcatgatgatggtggttgagcataacagcatgcttcgtcatatgtactcaacgacgaggtatcagtgatgccgcaaaaatcaaaacaggaggtgtggcaggccgcgcagattgaaggtgttggccacttcatagcagcaatcgccaaagcctttcctgatgcgatcgaggtggttcacgttcaaagcaataactgtaatgtttggtgttatgcgaaaactgatgtacaatcatctcatcaatcatcacccaccaccctttaacccgcttcggcgggttctttttttgccttatgcaccatggtgtagaatctgatacaatatcgaataacggaaaaatagcggaatattgataggttttatctatggctaaaaaactattcagtagcgaaaatcaaccacaaaataagcgcgggaaagacaagcgaaagctgcttgtagaggctcttgagcgcaagggattcagcgaggaaaagctgtacgataccattattgaaatggcaatgattgagcgcgataccgcgatgatgaaagagcttatcgtgcgatttagccccctaccaaagcctgtggcccctgtatttgaggttgatttcccggatgatggaactccggtagagaagattgatgcagtcattcgcggcattgcatccggcattattcccgccgatatcggtaagatgtttgccgaagttattaagaccggccttgatgtcgcggaagtaacagagcttgcggcgcgccttgagcgactggagaagttactggagcagcaacagtaactgatttataataatcaatacggctagggggcacccgaaaagcgactcatcaccgcctgccgcatcccaccaaagatgaccctgatgaggaaccaaaatgatcactcacgaagaactgattcaagtaatgacgtatgacccacaaactggtgttttttcatggaataaaacaaggcatggaataagaaacatggataatgcggggtgcgtaaccaagcgtggctatgtgaatatatacattaactacaaaaaataccttgcgcatagattagcgtggttttacgtttacggggaatggccttcgaagcaaattgatcacattaacggcgataagtctgataacagaatatcgaacttaagactggctaatggctctgaaaatcaactaaacagatggatagactcaaggaatacatctggtattaaaggtgtttgctggcataaaaataacaagaaatggcaagctagcgcatcacttggtggtaaggagtattatcttggccaatatgtaaacataaaagatgcggagaaggctgtggttgattttagggagaaacatcacggggagttttgtaaccatggctaggaaaaggctatcaagtattgcaatagaaaagctcgagcaggcggttggaaactcaactgcaaagcctgagtccgctgtgtttggcattgttgataaacttcttgccgatggcacgccaaatgttatcaagcgacttaaaatgactcaggatagtgtatcagagacaactgaagagccaacaatattaatccctgaacgcatggagcttttgctttatccgcgccggtttaaggtcttctatggcggaaggggcagcggcaaaacggctaacgtcgtttcctatcttatcgaaaaggcaagattcagaaattgcagggttggctgcttccgggaaattcagaactcaatcaagcaatcaagctacacagagcttgttgatgaaattaacagaaaggggcatgcgcatgaatacaggtgcgtagatggcgagataacacactacggcacgcggtcaaggttcgtgttccggggcatgtggcgcaacatcacggccatcaaagggatggctgggcttaccgatgtgttctgcgaggagtcggagaacattagtcaggtgtcatgggatacactcatccctacagttcgcgcctctggctctgaaattattattgtttttaaccccaatcgggaaaccgatcccacgtggacaaactttgttgagccgtatgtggataagatggttgatgggatatatcaggatgatgatattgtcgttgtgaacgttaactacatccataacccctggtttaccgaggaacttaaacagcacatgaaccagatgaaggcggttgattatgaccgctatctgtgggtttatgaggggttattcaaccggcgttcagatgaagctgtgcttgggggtaaatggcagactcttgattttgagccgtcgccagattggggcgggccttactatggtattgactttggtttctcgcaggatgctacggcagcaactgaatcttatgtcgaggatttgggtggcggaagaagaaacctgtatatctaccgcgactttgcaaaggttggtcttgagataactgatacgccagaagctatgcgactggcattcccgggttcagaaaaatacagatggtatggtgactgcgcaaggccagaaacaataagccatataaagcgctcaggatttgatatccatccgtgcgcaaagtggcctggcagcattgaggacggaatcacatggctcaggggttgtgacaggatttttgttcatgaaagatgtaagactgtcattgaggagtttactctttacagctacaaagtggacaagctcacgggaaatatacttcctgatatcatcgacaagcacaaccacgccacagatagtttgcgctatggccttggcgatcacattgtacagcgcggctctgggtggattaggcggagcaggagataagaaaaagccccgataaaggggcgatctattatctcaacttgaacaatttttctactgacggctttgaatggcctgacctgccattggcgcttaggctgctttttacatcaaactctgcaatgcattcaaagtcacctggagctttatattcactgatataaacatcgcatcttcttgataaattcctagtccaatcccaaaaatcatcattattaaacgaatccttgtaaccagtggtgccagcatacggagggtcgcagtacacaactgagccactctctatttgcatctcatcataactaagactagagaaaatgacgccttttaggtttttaatttgctgggctgcattctttattgcttcggcctggtaatccctcatgccacatcttgtttctactattccagcatacccaccgaaccatttcccgctgtacgagcaagctattccagcccatcctataaggtggtcatcaccctcgagattcttgagattcgcatattcatctctgcttataaacttaggattccatccggcgcatagcgccttaaatgcagcaataacgtacttattactgtcgttagcaaatcttgctcttgcatctctgacgccatcaatcatattcatgccgccagcaaatggctcataatagttcctaccaccagtattaagtaaagggatgattttatttttaagtcttgctttgctgcccatgtatttcatagataagcctcatcagtagaaaacaataatctacatcaaccacgaatcaacgtcaacatttataataaattatttgtaaagccagcaatggaccaggcatttccgatggcgcgtaaggctcgctggcatgctgactcatcaaggccggaaaccatcagtcacatcaagcgcgctggctttgacattcacccgtgcaacaaatggcccggcagtgttgaggatggcgttacatggctcaggggttgcgacaacatcatcattcacgaccgatgcgcagaaatgaaaaacgaggctgcgatgtatagccacaaggtcgacaagaacaccggcctggtgctgactgaaatcgttgataaatacaaccactattgggatgctgtgcgctatgcgttaaatgactatatcgtacagcgcggctctgggtggattaggcggagcaggagataagaaaaagccctcattagagggcttatttttataatgtgctctgagacctttttcctagttcgatgacgcaagccattgcagattctatggtgttgaactcatacagatgctttttatcttccatgacatagaacattaatcgtccaaatttatttttctttgcgctaaattgaatatctttcatctttgctatctccgctaatcaacttgatgaatcaaatctacatcagcaaacaatccacgtcaacatttataataaattatttgtaaagccagcaatgaatcccggcattgcgcatggctgcgtaaatcacgtcgtcagacacgactgccattgccactctgtctgcgtctatctgctggtgcgatgccatgatatcatcatagaaaatatcgttagcatgcagccactcatacgcatgctttgctctcatgataagcacatcgtgaccggcagagtaaagcgacttagccagcgctacgttgccagcaatatcatttccttcagcatcacgcagcacgccatcaagctcgaaaatgacacatttcataagatttctccgagaggtttcattttaatctacgccatgctagaatctacgtcaaggcgcattgacataactacatcaccggggcatcatgaaggcatactcatctttttcgtgggagcagaaggaaaaaatatactcactcgcaagagctggtgtgtctgatgaggcgctgtgcgaaaggtacgatgtggatgaggctattctgctgcgcatgtatgatgaagtgctgtgtgagttgcagcggcgccgtggttatagtggcctgaagacgattaatgatttctttcggaatgttgatttaaataatggtgaggatagtgaggatggtgatttgtgagagatattgtatttatggttatggtgaagttaccaacaatattcgccatcggtgcggctgcttggctggcattcaataacaaggaggggtggggttggtttctttttgttgcggtgctgataacttcatccgttaaaattgatgattgaggtggtgatgataaagaaaaagctgcaaatgaagatgcgcaaagccgcaatggagaagtacacaaggaagattgatatcagttttattgatggcgttggcatgtacaatcacgcatgccatcttaatgcggtaaatcgcgcaagagcaggaaacagtgccgccgtggttgaggttgttatgattaatgatgactcggttacagcgcattacatcaacatgcaggaggatgggaaatttgttgattacacgcttggctggcactggtcgggcgctgattacaggtttgtgcgatacgttccattcactgagtggggagatataacaagttcgcttgagctcctcaaggcagaactttgtaagccagtcagcaaatggatgcgcgcctttatgttgactaataacgaaatgtgttgaggtgatttatgattattgaagatgaaaccaaaacgccaatgtgcgaaatagctattcggtttgactctgaatcagtgattacgcaggggcatgacactattattgtcgacaaacgccaggctgcgcagcttatcgaagtcctgcaacgctgggttgatggcggggagattgagtgatgagcgtttatttttaccgtggtcacgcagagcgacacggaagcactgagagcgctggtagtttttgcggcgtcgttgtggcaactgatgctcttgccgggtatgagtcggcaatgagagagcagattaagtcaattagattgataaccgactcctgcgcagctaatttctctgttatttttgacaaattcgaaaaggtagagtgatgaagcgattccttttttcatggttatacctctttgtgatgtacatgatattccttgctctgtccttcccggtctgctggctcatcaaatggcagccgccgatgctgagcgatatcatgaacatcagcgtgctgcgcattactgtatttctgctggttgcgactatggttggcgcattatttcctagtagagttgattgaggtgaagtgatgtcgtatttcttcctgatattcgtaatcacaagcaacacgtccaatatgcaggtggtgccaatgcaaagcatggagcagtgcagtgcggccattacggcgatgaaaatcgctgagggaagacggacgtggcgtgatgtaagtacaaatattaacaatttgcaatgtgttgaggtgaagtgatgacaagaaaagagattcatgatgtggcggttggttgcaggaagtggattgaggagatatggtttaagcctggattcagtggaaagcgctataaattgcacgccaaatgtcgcggtttggttcttggggatagaatagagcttgctatattccataacaatgaccaggccctccaagagagagcctttggtgactgataccatgctataatcccatccatgcgatgggattttttatggtgacgaaatgtcaaagttagaggcggtaaacgcctatattcagcagcgagtggcgaacaataacaggctcatagagcggcagcgtcgggagcttggcgggaagaatatcgaccacaaacacgacaggctgtggctcgaatgcggctaccctgaagaaatcaccgccgagatgttccgccatgcctatgagcgctatgcaccggcagcagctggcgtcaatcgcgtactcgataagtgctggcagactccgccgcaaatcctccaggaaggcgccgatgataaggccagcactccgtgggagaaagcagccaataagttgtttaagcgtgctgcgccattcatcaaggatgcagaccgccgcaacctcatcaatcgctactccggcctcatcctgcaaatccgtgacggaaagcagtggaatgagccggtagacaccacgaaaacaaaacgcatcaaggatgctgccattgtccgttatattccggcgtgggaagagcagctccgcgtcagtgaatgggaaaatgacgaagccagcgaggactatggccagccgaagatgtacgaatatcaggagtcggtagtcggcgcctgcaacagcgacggaaaaccaacgcgttccctgagcattcaccctgaccgcattatcgtatttgccgagggcgcgatggatggctctatttattccggcgttccgctcctgcgtgccgggtataaccacctcatcgacatggcgaaagtcaccggctcaagcgcagaaggcttcctgaaaaatgccagccgacagctcaacgttaattataataaagacaacgtttccgctcagtctctggcgcagcaaatgcgcgtgccgctggaagagttggcggatgtcctcaatgaggatgtggcgcgcctgaatgaggcgattgacgcggcgatgttcacgatgggtgctgatgtcaaagtgctctcagtgacgccagcagacccgagtccaacgtggactattgcagccaaccagtttgcggcatccatcaagaagccattcaccatcctgtttggtcagcagactggccgccttgcatccgatgaggataaaaccgacgacgccatgagcgccaaacagcgccgcgaggactggctggattacatcatctcggtattcattgaccggatgatttccttcggcattctcgataaagcgccagagagcggttattactgcaaatgggatgacctgcttgcaccttccgagctgaataaggcagacctgctggtcaaacttgccgctgcaaacaaatccgtattcgacgcaggccagatggccctgatgaccgctgatgagatgcgcggcattgtcggcatggagcctctggaagagcagcttcctgacggattgcaggagggtcagcagcagcaagaccagcaaccgcagcaagaccaacagcaggaccagaccgatgcacctcctcaaaattaatgcccggcttccgcagccaaaattaagcatgagcctgacagacccactcggcgcagtgggtcgcgtcaataagatggtgcgcgatgttgacgccagatatgtgacgctaaaatctcaggttgccgggttgttcagcaccattccagtggcgaccggcaatgctgaggctggaaattattattatgatttctccgcctaccgcgcatcgacattctttgatgaacttcagcgcattcttgatgatcagctgctggaaggcgatgacttcacgcatggcaggatgtgggcttcatcctacgtcagtgacgcaatgtacgccggtacgcagaaggcaaacttagacctgagcgacctgtcgtcggcatacaaagacagcaggccgcttgctgaaatactgtactctcagccgtatctagacaggcttcagcttgcgtacacgcgcacgtataacgattggggtggcctttcagattacacgcggcaacaggtggcggaagtcatcactgctggcattgcaaacggcgatgcgccaggagtcgttgagcagaaaattgccgaccgcatggatgtgtcgcgcagctatgctcgctcgatagcacaaacagaaattaccaacaccctgcgtgaagccaatcgccgggaagtgaaagaggcacaggtgacactcggcatggataccatcatgctgtggcagtcggcactcatgaagactacccgcgttaatcacgccgcacgtcacggtaaatactacacaccagaagagattgatgaattctacagcgaaggtgctaaccgtcgcaattgccattgcagccagacccctgcgcttgtgatggatggcaagccggtgatactcgaaaggacgcaggagaaactggataaacagagagaagcgtggcagggagcacataaaaaagccgcctgatggcggcttgttggttatttttctgcaccaagtatcgctgatgctgcaaaccatacatttgcgataataaaatccacatcactctttgttgccactgagaatgcgaagtaaagaacaccaataatgagcgcaaccaggcatttcattatcaatcctccagcttcacgccgcgaactttaccggctgcgatggcgtcgtaaattttcttggcatgataaaattcgtttggtgtgtcagcaataaactcaggcagccagtaatcaatatcctcaacagcagcatcgcgcctcttatcggcttctgagctggtggggcggaattgatagttttcccattccagtgccaccgcatctttacccgcccaaccaaatgccacaccacaatcaatggccacgcagcggaaattcatccactcagcagaatctccgtgccggaatttggcttcgcactcacacccaacctgaggcagcccttctccaccccacgccagcgcaacatcctgcccgatgcactcattcaggtctgattcagcatcagattctgtgataccagcataagcatcccatgcggcagcgcgtacctgttctgatttcgtcggcttatgcaggctgtaggcgatgatgtctccccctgagttatcacttctccagaatggatatgatgcataaccacctgcgaaatgcgctttctgcgcatattccgtgcgaccattccttagcttgacatcaacaagaactccattttcaatcgggcattcaccgccaccccactcaatccagccttcatttttggcagccagcgcggattcgtactgttcgcgggtcacctcttcatcgctgtcctcgacctcaatatccgtgtcgattgtccattttggcgggcagccattattcttatcccagaaatatagcgtaccctcaccagagagaaacccggcgccaatggcaccatctggccacccgccacgcttcggaagttcttcaaccaaaatatcaatcagcttcatttcttatctccgttataaatgcttttcagttcacccattacattcagccatgctgcatgctcatccattccgcgcattaccagcttaacgtagcggttgcgggccttaaacatcaggcgcgggcacattacaagtcacccatgcttgatacgcaaagtgcaattgttattgccttgatttcttttggtgtcttgttcggcattgagtaggccatcttcactgttgcaccaagcaccttgttggcatccacgccgtactcagggctttgcgctactgccattgctatgctctgaggtacgccaggatcacgagcatctgccgccgcgaatccaacctcaccaaccttgtcgcatacctcaccagccgacgcaccaaaggaagacattgcgataattgctactgcgattaattttttcatttctactctcctgtgtttgtgtaactacatcatcgcccatgattcaatctacgtcaatatgattatgataaaataatctgcattaaagtggaggcactatgaaactatcaacgcgcggaaagaatttaattaaatcttatgagggactggttctcgcggtctaccctgacccggctaccggcggcgctccgtacaccgcaggatatggccacaccgggagcgatgttaagccgggaatgaaggtaactcaggcaatggctgacgcatggtttgataaagacgtagcgaaatttgaaagcggcgtctcgtcactcgtcaccgccccgacaactcagggccagtttgatgcaatggtgtcgctggcctataacatcgggcttggtaactttggcaaatcaactctgctgaaaaagcataacgcccgctgctacacctgcgccgctgaccagttccgggtgtggaatcgtgctaatggcaaggtcatgaacggactcaccaagcgccgcgcagctgagcgtgaggtatacatgtcatgaagcgcctcagtaactggcttatcggcatttgggcgtcattctgttcgctgattcagctctggcctgacgctatggttcatgtatgggcattcatgccggaagacttaaagtctgccattccgccgattgcagtcaaggccatcagctacagcattctcgttgcctcgctgcttgggaaaatgcatggcatgaagaaagagattaaggcgctgaaaaatgattctgcaaatccttaaagctaactggaaggttatagcggctattatcggcgccgcacttctggcgctgattatctacggaaagtgggtcaattacgggaaggcgaaatataattctggatatctggccgccgtagaggcgcagaaggtcaaagacaaagaggcaagcgaacaacatgagcaagacaaaaagaccatcgagcaggaagcgcaaggccgcattgatgccgcgcgtgctgatgcttccgctgctgctgctaagtctggcaggttgcagcaacagctcgccacaatcagaaagcagctcctcgattattcccgcactgagtccattggcaatccagcctcaaacaccggagttttgcttgccgacgtgctcagcaaatctgtcgaaagaaacagacaactggcagaatatgctgactcagcaagagaagcgggattgacttgtcaggcgcaatataactctctgaggtcagttaatgctaaatagagagaagcgcgaggagtatgacggaatggcggccaatgtggcgctaggcagggccggttatcaaccagcacgcaaaagccggtacagcaagtcagcaaaagatgaatatggccctgcgcctcaattcctgtagcaataaaaaagccccataaggggcttggcttggaaaactaaacaacgaagccgatattttcaccatcgagttttgcggcaatttcaacctcaataatcatggtggcaatctttcctctcgattgcgtgctggtgtcagttttcaccacgccgccaacaatcctcccatcctggtccaccacttgcaggcgtccgtcaataatctcctgatgtagccagattttttcagggtctttcgctgcttgtactgtcattttaaatcctcatagagtggtttcatctcatagccaaacatggctgcattttggtgctcaacactaccagcaaacgccagatagcggcgaccacgattgctggtgatgatgtaggcctttggtactctattctgctttaccgtcattatttaccagcctcctctgtcactttatcattggcggcagcgcgaaacagcgtcgcggtcagataaaatccaccaagccagaaataaccaagcgcgaacattactgctatttcgcaaaatgtagtcacaacctggtatttatgatgaatccatagcggctttttgtagcgagcaacggatttatcaagcaggtctttgcttgacagtaagccaactgatgcaatgattgacgcaatcgacatgaaccagaaaaaagccacagccatattgtatgcatgcacattctgcataaataggccgaagtaaatcagcggccacgtcaggaatatatcccatgcgatgtttttcaggagtcttttcattttgataacctcgcccagcctttacctttcacgttataaacaagccccttctttttcagtgcctgcattcttctgtcaaggattgtgatatttttaattggtgaaatgtcgaatacctcaaaccaaatcgacccgatatctacaggacggattgaatcatcaagacggcgcagaattgcatcgtcaagttcatcataagcacccatcactttacctccccgtttagttcgttaacaattaatgttgcatagccagcaatgtctttccagctatcgtcgtatgtcgggtcgccattcaggatgcgacagattttatgctgaatcatgtcgagtgcttctttctggctcgctgtcaggttattccagccatcaacgtcgcgcatggtgtctttcagtgactgcatgatttctgcaccgtctttgaatttcccgtagcgtttgcctcgctcggtgatgatggcttctgtggagttggcttctgtggagttggtgtgcccattcaagtcatcatcagttactggctcacgatgagcgataacaatatcgccagacttttcgatatccttatctcgccctgcataatccgcgccgaggtagtggatttttccactggttgctgattttacagcaagaacggcatcttcatgaccattaaaataatcagcacttcccttcaggtatttgtatttcatcactcacccctcaatgtaactttgtttttctcatccacgctgaagtgttcacgcacaaacgcatacatttcttcagcgctccattcccgaattgctacatagcagtgcgcgtaatatctgacatctcgcaggcttaacggctggcgcttagcgataatctcagtcaatacttccagtggttctttgcgttgtctcgccatctcttctctcctcgtaaaatagtattgactaatctacgtcatctagtcaatacttactggcgtagattgtatcatagttgcgaggagtggtgtggaatgaaaaagtggcaggaggtgacagaggttcataagcgcgattgccgggagactctgcaaatgcttaatgtgccagagtcaataattaaatctatcgagcagcgcattgacctggctgctatggaggcagcccatgaagccgaggaagcgcaaatgttgtcatggatgggcagaactctaccggtcgttttacatcgtggtaaaagtaccgattgaagatgatgacgggtatctgcacaaccatagtcaggtgctcaaatattatggcgttcactacaaagtgctgatggagagaaaaaatgactactgatcaggtgtacgaaaaagaattgctgaacaatctggaagaacttgaccgcactcgcgcatgggttgaaagcgaattgcacgaggttcgcaaccgcatgcaacggcaggttaaccgcgaaattatcgagtggcgcgaagggcgcccgcatttcagcaatattggtgaatgggtggcgaaatgaaaccaatgatgaatgatgatgggctgctggagtgtccgttttgcaatagcgatgatgtgtatcctgactctgatttagaggggaagaagcattttatttggtgtgggaattgcggttgtggaacaggagtaagacctaacaagtcatcagctgtgcgcaaatggaatacccgcaacggccacctctataccgctgacgactacaaacaagatgcagtggagcgcgcaaatggactttaaaacgcaaatactcaccgtgatagagcgctgcggcggtgcaaccaatgccatgatacgcaagcagactggcatgacaaaccgagccagcgttaccggctatctgattgaactggagagcatgggatttattattaaagaagagagtgtcagctatggcaggcgctgctttaagtatttcctcaatcccggcaataccgcgctcgatttggcaattcagacgtatcttgaggcgaatcctgggcgcaaaagcaagcagatagcagaggctgtaggcgtcaactacaccatcctcaaggcacgcatgcgctatctggcaagcattggtcaggttgaccgtgaaatgcttcccggcggcgcatggaaatattactggcaggaaatcatcccgtttggaatgagccgtgacaggatgatgtttgaaaagctgcttgcttgggcgcgccagtcatgtgggctgtaaagcataaatcaggaaccgtgatgtttgtcaccaattgtgaacgcacggccaataatcgcagagaaatggggtggatagtggaggaagtgaatgtgagcaaaccaaaaagcgcattaattaaaattacatggcatgacgacacggttagccagtggcatgcagattcattcagagagggtgagtactccattgaaatgaatattggtggatgcatcgtttgcatcccctggaggttatacaaagatggcgaagttaaacatttggatgtggagtcgtaaatgaaactacaacttaacgaaatcatggaagcaacaattagcgaactggatgacattgatatgacgcttgcctttgagattgaggctattgagcgccagcttgccggtaatcatgatgcgggcagagtatggagagagaaggccatgaaagcgcgtgaccatatgaaacgcacccgcgcactggttcgcactcgacttgataagctctactacggcgaagaaagaatgttgcacggcgccattctggctgaaatccgcaaaacgatgcctattgggaaattcatggatgcagtaaaccgcgcaaaaattaactgcggaatgctaaataagaatagtcctcaataaatcttcatccgtggctgttaccttgcattcaggaggtagcagccatgccaatcatactgatatcattctttgctactcttttcgcttttaccgcatctccgctttaccttctcgcgtccgtttcgtggtgcatattcatggtgtgttataatccgggcataaagtaagcgcggagaaaggtcatgattgtcaaaattggcgacaagtgggtcgttaaatctaaggatggctcgcaccagtttggcgagtacgacaccgaagaggcggcgaaaaagcgccttgctgaggtggaggcattcaagcacatgaataataaattacaggttaacatcctgtacaccatcaactcggccagcaacatcagtgaaaaaatcattgatggcgatccgcattatgtcatcaagaatgttgtgccggtggtagatgatattgtcatgaacggcggcctgtaccctggcgatgagattaaaaaatcattccatggtctggatggaaaaccggcgccatatgaccacccgaagattgatggcaaatatgtgtcagcaaacatgacgcgagccgccaatcagttcagcgttggtgcatggattgagaactcatctcatgacggcagcaaagcactggtagacctttatattaacaaggtggtagctgagcgctctgataaaggcaaagaattgctgtcgcgcattgacggactcaaagttaacagcgccgatgctgaacctgttcaggtgtctaccggtctgttgctcaaccgtgagcaggcatcaggaacttctaagggcaaaaaatattcctggattgcccgaaatatggagtgggatcacctcgcaattcttccgcctggcattcctggtgctggcggccctgctgatggtgtcggcatctttgctgctaacggcgaagacattgagcgtgttgtagtcaaccttgaggaatcggcaatgccagacgaaagtgcaaacaaaatcaaatggtggcagcgtgccattaatcgcctgaccggtaatcagctgtcattcgctgatattaccgcacaactccacaatatcatcaaggccgatatgcaagccgactcgtggccctatatcgtcgctgtttatgataattacttcggcgttgagattgacggcaccatttatatgcagtcctacatcgtccgcgaggatatggtagaattagtcggtgaacgggttaaggctgtttataagacagagcttgaaccggtaaaaacaactcaaggggaaatctcaatgactaacgaggaattacaggctgtattagccgatgccctcaagccggttcaggaatcgttgaccgcagtcaaccagaaactggccgatgtggaggcgcaaaacaaaactctgcgcgaccagctgcaagccaatgctgcgcaggaagagaccgcaatgcgcgccgccattatggctgagctgaagctgccggaagttgccgttaatgcgctgactggcgaagcactgcgtgaaacctatgcactcaccagtaaagcggctccgatttccggcgggttccagccgaaccgtgccgaagaagattttgatatggaggcacctgaataatggctactatccgttatggcaccatcatcggcggcccggcccgcaaaaacgacccgcagttgcgcgaaggtctgatgaacgtcgccctgcaacctggcgcactggtcgacttcaactcctctgacaaaatcatcgcgcatgcgactgctggcggtcatggtttcccttacgtcctgcaacacaactatgttggtggcggtgacgtgagcgaagctgtaccggcgaatgctaccggcatggcagtacagtgcgaatttggcgtaacgtatcacgctctggttgcggcatcatccgcgctggtaaaaggtactccgctggcaagcaatggctccggcgcgttaaaagtggctggcacaggtgataaaatcctgttctatgcgtatgaagcctacaccgtagcatctgatggcgctgaactcgttgcagttcgtcgtgctggcaatgctgcaatgcc